European Patent Application EP 4 261 225 A1, published October 18, 2023. Title: Anti-PD-1 Antibody and Use Thereof. Applicant: Eutilex Co., Ltd. The sequence listing filed with the application follows.

SEQUENCE LISTING (58 sequences)

SEQ ID NO: 1 - protein, 8 aa, Artificial Sequence
  H-CDR1
GFVFSNYD

SEQ ID NO: 2 - protein, 8 aa, Artificial Sequence
  H-CDR2
ITIGGGTT

SEQ ID NO: 3 - protein, 13 aa, Artificial Sequence
  H-CDR3
ARWVYDPLYAMDY

SEQ ID NO: 4 - protein, 13 aa, Artificial Sequence
  H-CDR3
ARRVYDPLYAMDY

SEQ ID NO: 5 - protein, 10 aa, Artificial Sequence
  L-CDR1
ESVDNYGISF

SEQ ID NO: 6 - protein, 3 aa, Artificial Sequence
  L-CDR2
AAS

SEQ ID NO: 7 - protein, 9 aa, Artificial Sequence
  L-CDR3
QQSKEVPWT

SEQ ID NO: 8 - protein, 8 aa, Artificial Sequence
  H-CDR1
GFTFSSFG

SEQ ID NO: 9 - protein, 8 aa, Artificial Sequence
  H-CDR2
IYSNGDYT

SEQ ID NO: 10 - protein, 13 aa, Artificial Sequence
  H-CDR3
ARYYGNYGGYFDY

SEQ ID NO: 11 - protein, 8 aa, Artificial Sequence
  L-CDR1
QSVSNDVA

SEQ ID NO: 12 - protein, 3 aa, Artificial Sequence
  L-CDR2
YAS

SEQ ID NO: 13 - protein, 9 aa, Artificial Sequence
  L-CDR3
QQDYSSPPT

SEQ ID NO: 14 - protein, 8 aa, Artificial Sequence
  H-CDR1
GYTFTTYW

SEQ ID NO: 15 - protein, 8 aa, Artificial Sequence
  H-CDR2
INPTTGYT

SEQ ID NO: 16 - protein, 10 aa, Artificial Sequence
  H-CDR3
ARGVRYYFDY

SEQ ID NO: 17 - protein, 12 aa, Artificial Sequence
  L-CDR1
QSLLDSRTRKNY

SEQ ID NO: 18 - protein, 3 aa, Artificial Sequence
  L-CDR2
WAS

SEQ ID NO: 19 - protein, 8 aa, Artificial Sequence
  L-CDR3
KQSYNLIT

SEQ ID NO: 20 - protein, 139 aa, Artificial Sequence
  VH
MDSRLNLVFLVLTLKGVKCEVQLVESGGGLVKPGGSLKLSCAASGFVFSNYDMSWVRQTPEKRLEWVAYITIGGGTTYYPDTVKGRFTISRDNAKNTLYLQMNSLKSEDTAIYYCARWVYDPLYAMDYWGQGTSVTVSS

SEQ ID NO: 21 - protein, 139 aa, Artificial Sequence
  VH
MDSRLNLVFLVLTLKGVKCEVQLVESGGGLVKPGGSLKLSCAASGFVFSNYDMSWVRQTPEKRLEWVAYITIGGGTTYYPDTVKGRFTISRDNAKNTLYLQMNSLKSEDTAIYYCARRVYDPLYAMDYWGQGTSVTVSS

SEQ ID NO: 22 - protein, 131 aa, Artificial Sequence
  VL
METDTLLLWVLLLWVPGSTGDILLTQSPASLAVSLGQRATISCRASESVDNYGISFMNWFQQKPGQPPKLLIYAASNQGSGVPARFSGSGSGTDFSLNIHPMEEDDTAMYFCQQSKEVPWTFGGGTKLEIK

SEQ ID NO: 23 - protein, 139 aa, Artificial Sequence
  VH
MDSRLNLVFLALILKGVQCEVQLVESGGGLVQPVGSLKLSCAASGFTFSSFGMSWVRQTPDKRLELVATIYSNGDYTYYPDSVKGRFTVSRDNAKNTLYLQMSSLKSEDTAMYYCARYYGNYGGYFDYWGQGTTLTVSS

SEQ ID NO: 24 - protein, 127 aa, Artificial Sequence
  VL
MESQTQVFVFLLLCVSGAHGSIVMTQTPKFLLVSAGDRVTITCKASQSVSNDVAWYQQKPGQSPKLLIYYASNRYTGAPDRFTGSGYGTDFTFTISTVQAEDLAVYFCQQDYSSPPTFGGGTKLEIK

SEQ ID NO: 25 - protein, 136 aa, Artificial Sequence
  VH
MECTWVILFLFSVTAGVHSQVQLQQSGAELAKPGASVKMSCKASGYTFTTYWIHWVKQRPGQGLEWIGYINPTTGYTEYNQKFKDKATLTADKSSNTAYMQLSSLTSEDSAVYYCARGVRYYFDYWGKGTTLTVSS

SEQ ID NO: 26 - protein, 136 aa, Artificial Sequence
  VL
MGFKMESQSLVLILLLLWVSGSCGDIVMSQSPSSLAVSAGEKVTMSCKSSQSLLDSRTRKNYLAWYQQKPGQSPKLLIYWASTRESGVPDRFTGSGSGTDFTLTISSVKAEDLAVYLCKQSYNLITFGAGTKLELK

SEQ ID NO: 27 - protein, 120 aa, Artificial Sequence
  VH
EVQLVESGGGLVQPGGSLRLSCAASGFVFSNYDMSWVRQAPGKGLEWVAYITIGGGTTYYPDTVKGRFTISRDNAKNSLYLQMNSLRAEDTAVYYCARWVYDPLYAMDYWGQGTTVTVSS

SEQ ID NO: 28 - protein, 120 aa, Artificial Sequence
  VH
EVQLVESGGGLVQPGGSLRLSCAASGFVFSNYDMSWVRQAPGKGLEWVAYITIGGGTTYYPDTVKGRFTISRDNAKNSLYLQMNSLRAEDTAVYYCARRVYDPLYAMDYWGQGTTVTVSS

SEQ ID NO: 29 - protein, 111 aa, Artificial Sequence
  VL
DIVLTQTPLSLSVTPGQPASISCRASESVDNYGISFMNWFLQKPGQPPQLLIYAASNQGSGVPDRFSGSGSGTDFTLKISRVEAEDVGVYYCQQSKEVPWTFGQGTKVEIK

SEQ ID NO: 30 - protein, 120 aa, Artificial Sequence
  VH
EVQLVESGGGLVKPGGSLRLSCAASGFTFSSFGMSWVRQAPGKGLELVATIYSNGDYTYYPDSVKGRFTVSRDNAKNSLYLQMNSLRAEDTAVYYCARYYGNYGGYFDYWGQGTLVTVSS

SEQ ID NO: 31 - protein, 107 aa, Artificial Sequence
  VL
AIQMTQSPSSLSASVGDRVTITCKASQSVSNDVAWYQQKPGKAPKLLIYYASNRYTGVPSRFSGSGSGTDFTLTISSLQPEDFATYYCQQDYSSPPTFGGGTKVEIK

SEQ ID NO: 32 - protein, 117 aa, Artificial Sequence
  VH
QVQLVQSGAEVKKPGASVKVSCKASGYTFTTYWIHWVRQAPGQGLEWIGYINPTTGYTEYNQKFKDRATLTADKSTSTAYMELSSLRSEDTAVYYCARGVRYYFDYWGKGTTVTVSS

SEQ ID NO: 33 - protein, 112 aa, Artificial Sequence
  VL
DIVMTQSPDSLAVSLGERATINCKSSQSLLDSRTRKNYLAWYQQKPGQPPKLLIYWASTRESGVPDRFSGSGSGTDFTLTISSLQAEDVAVYYCKQSYNLITFGQGTKLEIK

SEQ ID NO: 34 - DNA, 417 bp, Artificial Sequence
  VH coding Sequence
atggactccaggctcaatttagttttccttgtccttactttaaaaggtgtgaagtgtgaagtgcagctggtggagtctgggggaggcttagtgaagcctggagggtccctgaaactctcctgtgcagcctctggattcgttttcagtaactatgacatgtcttgggttcgccagactccggagaagaggctggagtgggtcgcatacattactattggtggtggtaccacctactatccagacactgtgaagggccgattcaccatctccagagacaatgccaagaacaccctgtaccttcaaatgaacagtctgaagtctgaggacacagccatatattactgtgcaaggtgggtctatgatcctctctatgctatggactactggggtcaaggaacctcagtcaccgtctcctca

SEQ ID NO: 35 - DNA, 417 bp, Artificial Sequence
  VH coding sequence
atggactccaggctcaatttagttttccttgtccttactttaaaaggtgtgaagtgtgaagtgcagctggtggagtctgggggaggcttagtgaagcctggagggtccctgaaactctcctgtgcagcctctggattcgttttcagtaactatgacatgtcttgggttcgccagactccggagaagaggctggagtgggtcgcatacattactattggtggtggtaccacctactatccagacactgtgaagggccgattcaccatctccagagacaatgccaagaacaccctgtaccttcaaatgaacagtctgaagtctgaggacacagccatatattactgtgcaaggcgggtctatgatcctctctatgctatggactactggggtcaaggaacctcagtcaccgtctcctca

SEQ ID NO: 36 - DNA, 393 bp, Artificial Sequence
  VL coding sequence
atggagacagacacactcctgctatgggtcctgcttctctgggttccaggttccacaggtgacattttgctgacccaatctccagcttctttggctgtgtctctagggcagagggccaccatctcctgcagagccagcgaaagtgttgataattatggcattagttttatgaactggttccaacagaaaccaggacagccacccaaactcctcatctatgctgcatccaaccaaggatccggggtccctgccaggtttagtggcagtgggtctgggacagacttcagcctcaacatccatcctatggaggaggatgatactgcaatgtatttctgtcagcaaagtaaggaggttccgtggacgttcggtggaggcaccaagctggaaatcaaa

SEQ ID NO: 37 - DNA, 417 bp, Artificial Sequence
  VH coding sequence
atggactccaggctcaatttagttttccttgcccttattttaaaaggtgtccagtgtgaggtgcagctggtggagtctgggggaggcttagtgcagcctgtagggtccctgaaactctcctgtgcagcctctggattcactttcagtagttttggcatgtcttgggttcgccagactccagacaagaggctggagttggtcgcaaccatttatagtaatggtgattacacctattatccagacagtgtgaagggccgattcaccgtctccagagacaatgccaagaacaccctgtacctgcaaatgagcagtctgaagtctgaggacacagccatgtattactgtgcaaggtactatggtaactacggggggtactttgactactggggccaaggcaccactctcacagtctcctca

SEQ ID NO: 38 - DNA, 381 bp, Artificial Sequence
  VL coding sequence
atggagtcacagacccaggtctttgtatttctactgctctgtgtgtctggtgctcatgggagtattgtgatgacccagactcccaaattcctgcttgtatcagcaggagacagggttaccataacctgcaaggccagtcagagtgtgagtaatgatgtagcttggtaccaacagaagccagggcagtctcctaaattgctgatatactatgcatccaatcgctacactggagcccctgatcgcttcactggcagtggatatgggacggatttcactttcaccatcagcactgtgcaggctgaagacctggcagtttatttctgtcagcaggattatagctctcctccgacattcggtggaggcaccaagctggaaatcaaa

SEQ ID NO: 39 - DNA, 408 bp, Artificial Sequence
  VH coding sequence
atggaatgcacctgggtcattctcttcctgttttcagtaactgcaggtgtccactcccaggtccagcttcagcagtctggggctgaactggcaaaacctggggcctcagtgaagatgtcctgcaaggcttctggctacacctttactacctactggattcactgggtaaaacagaggcctggacagggactggaatggattggatacattaatcctaccactggttatactgaatacaatcagaagttcaaggacaaggccacattgactgcagacaaatcctccaacacagcctacatgcaactgagcagcctgacatctgaggactctgcagtctattactgtgcaagaggagtacggtactactttgactactggggcaaaggcaccactctcacagtctcctca

SEQ ID NO: 40 - DNA, 408 bp, Artificial Sequence
  VL coding sequence
atgggcttcaagatggagtcacagtctctggttcttatattgctgctgctatgggtatctggttcctgtggggacattgtgatgtcacagtctccatcctccctggctgtgtcagcaggagagaaggtcactatgagctgcaaatccagtcagagtctgctcgacagtagaacccgaaagaactacttggcttggtaccagcagaaaccagggcagtctcctaaactgctgatctactgggcatccactagggaatctggggtccctgatcgcttcacaggcagtggatctgggacagatttcactctcaccatcagcagtgtgaaggctgaagacctggcagtttatctctgcaagcaatcttataatctgatcacgttcggtgctgggaccaagctggagctgaaa

SEQ ID NO: 41 - DNA, 360 bp, Artificial Sequence
  VH coding sequence
gaggtgcagctggtggagagcggcggcggcctggtgcagcccggcggcagcctgaggctgagctgcgccgccagcggcttcgtgttcagcaactacgacatgagctgggtgaggcaggcccccggcaagggcctggagtgggtggcctacatcaccatcggcggcggcaccacctactaccccgacaccgtgaagggcaggttcaccatcagcagggacaacgccaagaacagcctgtacctgcagatgaacagcctgagggccgaggacaccgccgtgtactactgcgccaggtgggtgtacgaccccctgtacgccatggactactggggccagggcaccaccgtgaccgtgagcagc

SEQ ID NO: 42 - DNA, 360 bp, Artificial Sequence
  VH coding sequence
gaggtgcagctggtggagagcggcggcggcctggtgcagcccggcggcagcctgaggctgagctgcgccgccagcggcttcgtgttcagcaactacgacatgagctgggtgaggcaggcccccggcaagggcctggagtgggtggcctacatcaccatcggcggcggcaccacctactaccccgacaccgtgaagggcaggttcaccatcagcagggacaacgccaagaacagcctgtacctgcagatgaacagcctgagggccgaggacaccgccgtgtactactgcgccaggagggtgtacgaccccctgtacgccatggactactggggccagggcaccaccgtgaccgtgagcagc

SEQ ID NO: 43 - DNA, 333 bp, Artificial Sequence
  VL coding sequence
gacatcgtgctgacccagacccccctgagcctgagcgtgacccccggccagcccgccagcatcagctgcagggccagcgagagcgtggacaactacggcatcagcttcatgaactggttcctgcagaagcccggccagcccccccagctgctgatctacgccgccagcaaccagggcagcggcgtgcccgacaggttcagcggcagcggcagcggcaccgacttcaccctgaagatcagcagggtggaggccgaggacgtgggcgtgtactactgccagcagagcaaggaggtgccctggaccttcggccagggcaccaaggtggagatcaag

SEQ ID NO: 44 - DNA, 360 bp, Artificial Sequence
  VH coding sequence
gaggtgcagctggtggagagcggcggcggcctggtgaagcccggcggcagcctgaggctgagctgcgccgccagcggcttcaccttcagcagcttcggcatgagctgggtgaggcaggcccccggcaagggcctggagctggtggccaccatctacagcaacggcgactacacctactaccccgacagcgtgaagggcaggttcaccgtgagcagggacaacgccaagaacagcctgtacctgcagatgaacagcctgagggccgaggacaccgccgtgtactactgcgccaggtactacggcaactacggcggctacttcgactactggggccagggcaccctggtgaccgtgagcagc

SEQ ID NO: 45 - DNA, 321 bp, Artificial Sequence
  VL coding sequence
gccatccagatgacccagagccccagcagcctgagcgccagcgtgggcgacagggtgaccatcacctgcaaggccagccagagcgtgagcaacgacgtggcctggtaccagcagaagcccggcaaggcccccaagctgctgatctactacgccagcaacaggtacaccggcgtgcccagcaggttcagcggcagcggcagcggcaccgacttcaccctgaccatcagcagcctgcagcccgaggacttcgccacctactactgccagcaggactacagcagcccccccaccttcggcggcggcaccaaggtggagatcaag

SEQ ID NO: 46 - DNA, 351 bp, Artificial Sequence
  VH coding sequence
caggtgcagctggtgcagagcggcgccgaggtgaagaagcccggcgccagcgtgaaggtgagctgcaaggccagcggctacaccttcaccacctactggatccactgggtgaggcaggcccccggccagggcctggagtggatcggctacatcaaccccaccaccggctacaccgagtacaaccagaagttcaaggacagggccaccctgaccgccgacaagagcaccagcaccgcctacatggagctgagcagcctgaggagcgaggacaccgccgtgtactactgcgccaggggcgtgaggtactacttcgactactggggcaagggcaccaccgtgaccgtgagcagc

SEQ ID NO: 47 - DNA, 336 bp, Artificial Sequence
  VL coding sequence
gacatcgtgatgacccagagccccgacagcctggccgtgagcctgggcgagagggccaccatcaactgcaagagcagccagagcctgctggacagcaggaccaggaagaactacctggcctggtaccagcagaagcccggccagccccccaagctgctgatctactgggccagcaccagggagagcggcgtgcccgacaggttcagcggcagcggcagcggcaccgacttcaccctgaccatcagcagcctgcaggccgaggacgtggccgtgtactactgcaagcagagctacaacctgatcaccttcggccagggcaccaagctggagatcaag

SEQ ID NO: 48 - protein, 120 aa, Artificial Sequence
  2B3W-T14-05 VH
EVQLVESGGGLVQPGGSLRLSCAASGFVFSNYDMSWVRQAPGKGLEWVAYITIGGGTTYYPDTVKGRFTISRDNAKNSLYLQMNSLRAEDTAVYYCARWRYDPLFAMDYWGQGTTVTVSS

SEQ ID NO: 49 - protein, 111 aa, Artificial Sequence
  2B3W-T14-05 VL
DIVLTQTPLSLSVTPGQPASISCRASESVTDYGISFMNWFLQKPGQPPQLLIYAASNQGSGVPDRFSGSGSGTDFTLKISRVEAEDVGVYYCQQSKEVPWTFGQGTKVEIK

SEQ ID NO: 50 - protein, 120 aa, Artificial Sequence; identical to SEQ ID NO: 30
  7C5-T15-01 VH

SEQ ID NO: 51 - protein, 107 aa, Artificial Sequence
  7C5-T15-01 VL
AIQMTQSPSSLSASVGDRVTITCKASQSVWDDLTWYQQKPGKAPKLLIYYASNRYTGVPSRFSGSGSGTDFTLTISSLQPEDFATYYCQQDYSSPPTFGGGTKVEIK

SEQ ID NO: 52 - protein, 117 aa, Artificial Sequence; identical to SEQ ID NO: 32
  8D4-T16-01 VH

SEQ ID NO: 53 - protein, 112 aa, Artificial Sequence; identical to SEQ ID NO: 33
  8D4-T16-01 VL

SEQ ID NO: 54 - protein, 117 aa, Artificial Sequence; identical to SEQ ID NO: 32
  8D4-T16-02 VH

SEQ ID NO: 55 - protein, 113 aa, Artificial Sequence
  8D4-T16-02 VL
DIVMTQSPDSLAVSLGERATINCKSSQSLLDSRTRKNYLAWYQQKPGQPPKLLIYWASTRESGVPDRFSGSGSGTDFTLTISSLQAEDVAVYYCQQQYDPPITFGQGTKLEIK

SEQ ID NO: 56 - protein, 14 aa, Artificial Sequence
  VH CDR3
ARWRYDPLFAMDYW

SEQ ID NO: 57 - protein, 12 aa, Artificial Sequence
  VL CDR1
ESVTDYGISFMN

SEQ ID NO: 58 - protein, 8 aa, Artificial Sequence
  VL CDR1
QSVWDDLT